European Patent Application EP 4 207 001 A1, published July 5, 2023. Title: METHOD FOR MOLECULAR COMPUTING. Applicant: DNA 2 ASCENDANCY AB. The sequence listing filed with the application follows.

SEQUENCE LISTING (6 sequences)

SEQ ID NO: 1 - DNA, 49 bp, Artificial sequence
  Synthesized DNA representing calculation elements
tctggtctgggatgtgaggtctggtctggagatagaggcagagtgtgag

SEQ ID NO: 2 - DNA, 41 bp, Artificial sequence
  Synthesized DNA representing calculation elements
aggactggtctgggatgtgaggactggtctggagatagagg

SEQ ID NO: 3 - DNA, 19 bp, Artificial sequence
  Synthesized DNA representing calculation elements
tctggtctgggatgtgagg

SEQ ID NO: 4 - DNA, 19 bp, Artificial sequence
  Synthesized DNA representing calculation elements
tctggtctggagatagagg

SEQ ID NO: 5 - DNA, 19 bp, Artificial sequence
  Synthesized DNA representing calculation elements
actggtctgggatgtgagg

SEQ ID NO: 6 - DNA, 19 bp, Artificial sequence
  Synthesized DNA representing calculation elements
actggtctggagatagagg